European Patent Application EP 4 273 159 A1, published November 8, 2023. Title: HUMAN GLP-1 POLYPEPTIDE VARIANT AND USE THEREOF. Applicant: Suzhou Alphamab Co., Ltd. The sequence listing filed with the application follows.

SEQUENCE LISTING (154 sequences)

SEQ ID NO: 1 - protein, 31 aa, Homo sapiens
HAEGTFTSDVSSYLEGQAAKEFIAWLVKGRG

SEQ ID NO: 2 - protein, 31 aa, Artificial Sequence
  N-terminal GLP-1 sequence in dulaglutide
HGEGTFTSDVSSYLEEQAAKEFIAWLVKGGG

SEQ ID NO: 3 - protein, 351 aa, Artificial Sequence
  GLP1R-muFc
RPQGATVSLWETVQKWREYRRQCQRSLTEDPPPATDLFCNRTFDEYACWPDGEPGSFVNVSCPWYLPWASSVPQGHVYRFCTAEGLWLQKDNSSLPWRDLSECEESKRGERSSPEEGAPGSMDPKSSDKTHTCPPCPAPEVSSVFIFPPKPKDVLTITLTPKVTCVVVDISKDDPEVQFSWFVDDVEVHTAQTQPREEQFNSTFRSVSELPIMHQDWLNGKEFKCRVNSAAFPAPIEKTISKTKGRPKAPQVYTIPPPKEQMAKDKVSLTCMITDFFPEDITVEWQWNGQPAENYKNTQPIMNTNGSYFVYSKLNVQKSNWEAGNTFTCSVLHEGLHNHHTEKSLSHSPGK

SEQ ID NO: 4 - protein, 275 aa, Artificial Sequence
  Dulaglutide/KN042 sequence/GLP-1-Fc
HGEGTFTSDVSSYLEEQAAKEFIAWLVKGGGGGGGSGGGGSGGGGSAESKYGPPCPPCPAPEAAGGPSVFLFPPKPKDTLMISRTPEVTCVVVDVSQEDPEVQFNWYVDGVEVHNAKTKPREEQFNSTYRVVSVLTVLHQDWLNGKEYKCKVSNKGLPSSIEKTISKAKGQPREPQVYTLPPSQEEMTKNQVSLTCLVKGFYPSDIAVEWESNGQPENNYKTTPPVLDSDGSFFLYSRLTVDKSRWQEGNVFSCSVMHEALHNHYTQKSLSLSLG

SEQ ID NO: 5 - protein, 31 aa, Artificial Sequence
  GLP-1-WY
HGEGTFTSDVSSYLEEQAAKEFIAYLVKGGG

SEQ ID NO: 6 - protein, 31 aa, Artificial Sequence
  GLP-1-WR
HGEGTFTSDVSSYLEEQAAKEFIARLVKGGG

SEQ ID NO: 7 - protein, 31 aa, Artificial Sequence
  GLP-1-WK
HGEGTFTSDVSSYLEEQAAKEFIAKLVKGGG

SEQ ID NO: 8 - protein, 31 aa, Artificial Sequence
  GLP-1-FY
HGEGTFTSDVSSYLEEQAAKEYIAWLVKGGG

SEQ ID NO: 9 - protein, 31 aa, Artificial Sequence
  GLP-1-FH
HGEGTFTSDVSSYLEEQAAKEHIAWLVKGGG

SEQ ID NO: 10 - protein, 31 aa, Artificial Sequence
  GLP-1-FT
HGEGTFTSDVSSYLEEQAAKETIAWLVKGGG

SEQ ID NO: 11 - protein, 31 aa, Artificial Sequence
  GLP-1-FN
HGEGTFTSDVSSYLEEQAAKENIAWLVKGGG

SEQ ID NO: 12 - protein, 31 aa, Artificial Sequence
  GLP-1-FS
HGEGTFTSDVSSYLEEQAAKESIAWLVKGGG

SEQ ID NO: 13 - protein, 31 aa, Artificial Sequence
  GLP-1-FQ
HGEGTFTSDVSSYLEEQAAKEQIAWLVKGGG

SEQ ID NO: 14 - protein, 31 aa, Artificial Sequence
  GLP-1-FE
HGEGTFTSDVSSYLEEQAAKEEIAWLVKGGG

SEQ ID NO: 15 - protein, 31 aa, Artificial Sequence
  GLP-1-FV
HGEGTFTSDVSSYLEEQAAKEVIAWLVKGGG

SEQ ID NO: 16 - protein, 31 aa, Artificial Sequence
  GLP-1-FK
HGEGTFTSDVSSYLEEQAAKEKIAWLVKGGG

SEQ ID NO: 17 - protein, 31 aa, Artificial Sequence
  GLP-1-FI
HGEGTFTSDVSSYLEEQAAKEIIAWLVKGGG

SEQ ID NO: 18 - protein, 31 aa, Artificial Sequence
  GLP-1-QN
HGEGTFTSDVSSYLEENAAKEFIAWLVKGGG

SEQ ID NO: 19 - protein, 31 aa, Artificial Sequence
  GLP-1-QT
HGEGTFTSDVSSYLEETAAKEFIAWLVKGGG

SEQ ID NO: 20 - protein, 31 aa, Artificial Sequence
  GLP-1-QS
HGEGTFTSDVSSYLEESAAKEFIAWLVKGGG

SEQ ID NO: 21 - protein, 31 aa, Artificial Sequence
  GLP-1-QE
HGEGTFTSDVSSYLEEEAAKEFIAWLVKGGG

SEQ ID NO: 22 - protein, 31 aa, Artificial Sequence
  GLP-1-YL
HGEGTFTSDVSSLLEEQAAKEFIAWLVKGGG

SEQ ID NO: 23 - protein, 31 aa, Artificial Sequence
  GLP-1-YT
HGEGTFTSDVSSTLEEQAAKEFIAWLVKGGG

SEQ ID NO: 24 - protein, 31 aa, Artificial Sequence
  GLP-1-YF
HGEGTFTSDVSSFLEEQAAKEFIAWLVKGGG

SEQ ID NO: 25 - protein, 31 aa, Artificial Sequence
  GLP-1-YI
HGEGTFTSDVSSILEEQAAKEFIAWLVKGGG

SEQ ID NO: 26 - protein, 31 aa, Artificial Sequence
  GLP-1-YV
HGEGTFTSDVSSVLEEQAAKEFIAWLVKGGG

SEQ ID NO: 27 - protein, 31 aa, Artificial Sequence
  GLP-1-YS
HGEGTFTSDVSSSLEEQAAKEFIAWLVKGGG

SEQ ID NO: 28 - protein, 31 aa, Artificial Sequence
  GLP-1-YA
HGEGTFTSDVSSALEEQAAKEFIAWLVKGGG

SEQ ID NO: 29 - protein, 31 aa, Artificial Sequence
  GLP-1-KRWY
HGEGTFTSDVSSYLEEQAAREFIAYLVKGGG

SEQ ID NO: 30 - protein, 31 aa, Artificial Sequence
  GLP-1-KRFY
HGEGTFTSDVSSYLEEQAAREYIAWLVKGGG

SEQ ID NO: 31 - protein, 31 aa, Artificial Sequence
  GLP-1-KRWYFY
HGEGTFTSDVSSYLEEQAAREYIAYLVKGGG

SEQ ID NO: 32 - protein, 31 aa, Artificial Sequence
  GLP-1-KRQN
HGEGTFTSDVSSYLEENAAREFIAWLVKGGG

SEQ ID NO: 33 - protein, 31 aa, Artificial Sequence
  GLP-1-KRQT
HGEGTFTSDVSSYLEETAAREFIAWLVKGGG

SEQ ID NO: 34 - protein, 31 aa, Artificial Sequence
  GLP-1-KRQS
HGEGTFTSDVSSYLEESAAREFIAWLVKGGG

SEQ ID NO: 35 - protein, 31 aa, Artificial Sequence
  GLP-1-KRQE
HGEGTFTSDVSSYLEEEAAREFIAWLVKGGG

SEQ ID NO: 36 - protein, 31 aa, Artificial Sequence
  GLP-1-KRYL
HGEGTFTSDVSSLLEEQAAREFIAWLVKGGG

SEQ ID NO: 37 - protein, 31 aa, Artificial Sequence
  GLP-1-KRYT
HGEGTFTSDVSSTLEEQAAREFIAWLVKGGG

SEQ ID NO: 38 - protein, 31 aa, Artificial Sequence
  GLP-1-KRYF
HGEGTFTSDVSSFLEEQAAREFIAWLVKGGG

SEQ ID NO: 39 - protein, 31 aa, Artificial Sequence
  GLP-1-KRYI
HGEGTFTSDVSSILEEQAAREFIAWLVKGGG

SEQ ID NO: 40 - protein, 31 aa, Artificial Sequence
  GLP-1-KRYV
HGEGTFTSDVSSVLEEQAAREFIAWLVKGGG

SEQ ID NO: 41 - protein, 31 aa, Artificial Sequence
  GLP-1-KRYS
HGEGTFTSDVSSSLEEQAAREFIAWLVKGGG

SEQ ID NO: 42 - protein, 31 aa, Artificial Sequence
  GLP-1-KRYA
HGEGTFTSDVSSALEEQAAREFIAWLVKGGG

SEQ ID NO: 43 - protein, 31 aa, Artificial Sequence
  GLP-1-WYQN
HGEGTFTSDVSSYLEENAAKEFIAYLVKGGG

SEQ ID NO: 44 - protein, 31 aa, Artificial Sequence
  GLP-1-WYQS
HGEGTFTSDVSSYLEESAAKEFIAYLVKGGG

SEQ ID NO: 45 - protein, 31 aa, Artificial Sequence
  GLP-1-WYQT
HGEGTFTSDVSSYLEETAAKEFIAYLVKGGG

SEQ ID NO: 46 - protein, 31 aa, Artificial Sequence
  GLP-1-WYQE
HGEGTFTSDVSSYLEEEAAKEFIAYLVKGGG

SEQ ID NO: 47 - protein, 31 aa, Artificial Sequence
  GLP-1-WYYL
HGEGTFTSDVSSLLEEQAAKEFIAYLVKGGG

SEQ ID NO: 48 - protein, 31 aa, Artificial Sequence
  GLP-1-WYYT
HGEGTFTSDVSSTLEEQAAKEFIAYLVKGGG

SEQ ID NO: 49 - protein, 31 aa, Artificial Sequence
  GLP-1-WYYF
HGEGTFTSDVSSFLEEQAAKEFIAYLVKGGG

SEQ ID NO: 50 - protein, 31 aa, Artificial Sequence
  GLP-1-WYYI
HGEGTFTSDVSSILEEQAAKEFIAYLVKGGG

SEQ ID NO: 51 - protein, 31 aa, Artificial Sequence
  GLP-1-WYYV
HGEGTFTSDVSSVLEEQAAKEFIAYLVKGGG

SEQ ID NO: 52 - protein, 31 aa, Artificial Sequence
  GLP-1-WYYS
HGEGTFTSDVSSSLEEQAAKEFIAYLVKGGG

SEQ ID NO: 53 - protein, 31 aa, Artificial Sequence
  GLP-1-WYYA
HGEGTFTSDVSSALEEQAAKEFIAYLVKGGG

SEQ ID NO: 54 - protein, 31 aa, Artificial Sequence
  GLP-1-WYFY
HGEGTFTSDVSSYLEEQAAKEYIAYLVKGGG

SEQ ID NO: 55 - protein, 31 aa, Artificial Sequence
  GLP-1-WYFL
HGEGTFTSDVSSYLEEQAAKELIAYLVKGGG

SEQ ID NO: 56 - protein, 31 aa, Artificial Sequence
  GLP-1-WA
HGEGTFTSDVSSYLEEQAAKEFIAALVKGGG

SEQ ID NO: 57 - protein, 31 aa, Artificial Sequence
  GLP-1-WL
HGEGTFTSDVSSYLEEQAAKEFIALLVKGGG

SEQ ID NO: 58 - protein, 31 aa, Artificial Sequence
  GLP-1-FL
HGEGTFTSDVSSYLEEQAAKELIAWLVKGGG

SEQ ID NO: 59 - protein, 31 aa, Artificial Sequence
  GLP-1-WIFL
HGEGTFTSDVSSYLEEQAAKELIAILVKGGG

SEQ ID NO: 60 - protein, 31 aa, Artificial Sequence
  GLP-1-WLFL
HGEGTFTSDVSSYLEEQAAKELIALLVKGGG

SEQ ID NO: 61 - protein, 31 aa, Artificial Sequence
  GLP-1-KRWYQN
HGEGTFTSDVSSYLEENAAREFIAYLVKGGG

SEQ ID NO: 62 - protein, 31 aa, Artificial Sequence
  GLP-1-KRWYQT
HGEGTFTSDVSSYLEETAAREFIAYLVKGGG

SEQ ID NO: 63 - protein, 31 aa, Artificial Sequence
  GLP-1-KRWYQS
HGEGTFTSDVSSYLEESAAREFIAYLVKGGG

SEQ ID NO: 64 - protein, 31 aa, Artificial Sequence
  GLP-1-KRWYQE
HGEGTFTSDVSSYLEEEAAREFIAYLVKGGG

SEQ ID NO: 65 - protein, 31 aa, Artificial Sequence
  GLP-1-KRWYYF
HGEGTFTSDVSSFLEEQAAREFIAYLVKGGG

SEQ ID NO: 66 - protein, 31 aa, Artificial Sequence
  GLP-1-KRWYYL
HGEGTFTSDVSSLLEEQAAREFIAYLVKGGG

SEQ ID NO: 67 - protein, 31 aa, Artificial Sequence
  GLP-1-KRWYYT
HGEGTFTSDVSSTLEEQAAREFIAYLVKGGG

SEQ ID NO: 68 - protein, 31 aa, Artificial Sequence
  GLP-1-KRWYYI
HGEGTFTSDVSSILEEQAAREFIAYLVKGGG

SEQ ID NO: 69 - protein, 31 aa, Artificial Sequence
  GLP-1-KRWYYV
HGEGTFTSDVSSVLEEQAAREFIAYLVKGGG

SEQ ID NO: 70 - protein, 31 aa, Artificial Sequence
  GLP-1-KRWYYS
HGEGTFTSDVSSSLEEQAAREFIAYLVKGGG

SEQ ID NO: 71 - protein, 31 aa, Artificial Sequence
  GLP-1-KRWYYA
HGEGTFTSDVSSALEEQAAREFIAYLVKGGG

SEQ ID NO: 72 - protein, 275 aa, Artificial Sequence
  GM-WY
HGEGTFTSDVSSYLEEQAAKEFIAYLVKGGGGGGGSGGGGSGGGGSAESKYGPPCPPCPAPEAAGGPSVFLFPPKPKDTLMISRTPEVTCVVVDVSQEDPEVQFNWYVDGVEVHNAKTKPREEQFNSTYRVVSVLTVLHQDWLNGKEYKCKVSNKGLPSSIEKTISKAKGQPREPQVYTLPPSQEEMTKNQVSLTCLVKGFYPSDIAVEWESNGQPENNYKTTPPVLDSDGSFFLYSRLTVDKSRWQEGNVFSCSVMHEALHNHYTQKSLSLSLG

SEQ ID NO: 73 - protein, 275 aa, Artificial Sequence
  GM-WR
HGEGTFTSDVSSYLEEQAAKEFIARLVKGGGGGGGSGGGGSGGGGSAESKYGPPCPPCPAPEAAGGPSVFLFPPKPKDTLMISRTPEVTCVVVDVSQEDPEVQFNWYVDGVEVHNAKTKPREEQFNSTYRVVSVLTVLHQDWLNGKEYKCKVSNKGLPSSIEKTISKAKGQPREPQVYTLPPSQEEMTKNQVSLTCLVKGFYPSDIAVEWESNGQPENNYKTTPPVLDSDGSFFLYSRLTVDKSRWQEGNVFSCSVMHEALHNHYTQKSLSLSLG

SEQ ID NO: 74 - protein, 275 aa, Artificial Sequence
  GM-WK
HGEGTFTSDVSSYLEEQAAKEFIAKLVKGGGGGGGSGGGGSGGGGSAESKYGPPCPPCPAPEAAGGPSVFLFPPKPKDTLMISRTPEVTCVVVDVSQEDPEVQFNWYVDGVEVHNAKTKPREEQFNSTYRVVSVLTVLHQDWLNGKEYKCKVSNKGLPSSIEKTISKAKGQPREPQVYTLPPSQEEMTKNQVSLTCLVKGFYPSDIAVEWESNGQPENNYKTTPPVLDSDGSFFLYSRLTVDKSRWQEGNVFSCSVMHEALHNHYTQKSLSLSLG

SEQ ID NO: 75 - protein, 275 aa, Artificial Sequence
  GM-FY
HGEGTFTSDVSSYLEEQAAKEYIAWLVKGGGGGGGSGGGGSGGGGSAESKYGPPCPPCPAPEAAGGPSVFLFPPKPKDTLMISRTPEVTCVVVDVSQEDPEVQFNWYVDGVEVHNAKTKPREEQFNSTYRVVSVLTVLHQDWLNGKEYKCKVSNKGLPSSIEKTISKAKGQPREPQVYTLPPSQEEMTKNQVSLTCLVKGFYPSDIAVEWESNGQPENNYKTTPPVLDSDGSFFLYSRLTVDKSRWQEGNVFSCSVMHEALHNHYTQKSLSLSLG

SEQ ID NO: 76 - protein, 275 aa, Artificial Sequence
  GM-FH
HGEGTFTSDVSSYLEEQAAKEHIAWLVKGGGGGGGSGGGGSGGGGSAESKYGPPCPPCPAPEAAGGPSVFLFPPKPKDTLMISRTPEVTCVVVDVSQEDPEVQFNWYVDGVEVHNAKTKPREEQFNSTYRVVSVLTVLHQDWLNGKEYKCKVSNKGLPSSIEKTISKAKGQPREPQVYTLPPSQEEMTKNQVSLTCLVKGFYPSDIAVEWESNGQPENNYKTTPPVLDSDGSFFLYSRLTVDKSRWQEGNVFSCSVMHEALHNHYTQKSLSLSLG

SEQ ID NO: 77 - protein, 275 aa, Artificial Sequence
  GM-FT
HGEGTFTSDVSSYLEEQAAKETIAWLVKGGGGGGGSGGGGSGGGGSAESKYGPPCPPCPAPEAAGGPSVFLFPPKPKDTLMISRTPEVTCVVVDVSQEDPEVQFNWYVDGVEVHNAKTKPREEQFNSTYRVVSVLTVLHQDWLNGKEYKCKVSNKGLPSSIEKTISKAKGQPREPQVYTLPPSQEEMTKNQVSLTCLVKGFYPSDIAVEWESNGQPENNYKTTPPVLDSDGSFFLYSRLTVDKSRWQEGNVFSCSVMHEALHNHYTQKSLSLSLG

SEQ ID NO: 78 - protein, 275 aa, Artificial Sequence
  GM-FN
HGEGTFTSDVSSYLEEQAAKENIAWLVKGGGGGGGSGGGGSGGGGSAESKYGPPCPPCPAPEAAGGPSVFLFPPKPKDTLMISRTPEVTCVVVDVSQEDPEVQFNWYVDGVEVHNAKTKPREEQFNSTYRVVSVLTVLHQDWLNGKEYKCKVSNKGLPSSIEKTISKAKGQPREPQVYTLPPSQEEMTKNQVSLTCLVKGFYPSDIAVEWESNGQPENNYKTTPPVLDSDGSFFLYSRLTVDKSRWQEGNVFSCSVMHEALHNHYTQKSLSLSLG

SEQ ID NO: 79 - protein, 275 aa, Artificial Sequence
  GM-FS
HGEGTFTSDVSSYLEEQAAKESIAWLVKGGGGGGGSGGGGSGGGGSAESKYGPPCPPCPAPEAAGGPSVFLFPPKPKDTLMISRTPEVTCVVVDVSQEDPEVQFNWYVDGVEVHNAKTKPREEQFNSTYRVVSVLTVLHQDWLNGKEYKCKVSNKGLPSSIEKTISKAKGQPREPQVYTLPPSQEEMTKNQVSLTCLVKGFYPSDIAVEWESNGQPENNYKTTPPVLDSDGSFFLYSRLTVDKSRWQEGNVFSCSVMHEALHNHYTQKSLSLSLG

SEQ ID NO: 80 - protein, 275 aa, Artificial Sequence
  GM-FQ
HGEGTFTSDVSSYLEEQAAKEQIAWLVKGGGGGGGSGGGGSGGGGSAESKYGPPCPPCPAPEAAGGPSVFLFPPKPKDTLMISRTPEVTCVVVDVSQEDPEVQFNWYVDGVEVHNAKTKPREEQFNSTYRVVSVLTVLHQDWLNGKEYKCKVSNKGLPSSIEKTISKAKGQPREPQVYTLPPSQEEMTKNQVSLTCLVKGFYPSDIAVEWESNGQPENNYKTTPPVLDSDGSFFLYSRLTVDKSRWQEGNVFSCSVMHEALHNHYTQKSLSLSLG

SEQ ID NO: 81 - protein, 275 aa, Artificial Sequence
  GM-FE
HGEGTFTSDVSSYLEEQAAKEEIAWLVKGGGGGGGSGGGGSGGGGSAESKYGPPCPPCPAPEAAGGPSVFLFPPKPKDTLMISRTPEVTCVVVDVSQEDPEVQFNWYVDGVEVHNAKTKPREEQFNSTYRVVSVLTVLHQDWLNGKEYKCKVSNKGLPSSIEKTISKAKGQPREPQVYTLPPSQEEMTKNQVSLTCLVKGFYPSDIAVEWESNGQPENNYKTTPPVLDSDGSFFLYSRLTVDKSRWQEGNVFSCSVMHEALHNHYTQKSLSLSLG

SEQ ID NO: 82 - protein, 275 aa, Artificial Sequence
  GM-FV
HGEGTFTSDVSSYLEEQAAKEVIAWLVKGGGGGGGSGGGGSGGGGSAESKYGPPCPPCPAPEAAGGPSVFLFPPKPKDTLMISRTPEVTCVVVDVSQEDPEVQFNWYVDGVEVHNAKTKPREEQFNSTYRVVSVLTVLHQDWLNGKEYKCKVSNKGLPSSIEKTISKAKGQPREPQVYTLPPSQEEMTKNQVSLTCLVKGFYPSDIAVEWESNGQPENNYKTTPPVLDSDGSFFLYSRLTVDKSRWQEGNVFSCSVMHEALHNHYTQKSLSLSLG

SEQ ID NO: 83 - protein, 275 aa, Artificial Sequence
  GM-FK
HGEGTFTSDVSSYLEEQAAKEKIAWLVKGGGGGGGSGGGGSGGGGSAESKYGPPCPPCPAPEAAGGPSVFLFPPKPKDTLMISRTPEVTCVVVDVSQEDPEVQFNWYVDGVEVHNAKTKPREEQFNSTYRVVSVLTVLHQDWLNGKEYKCKVSNKGLPSSIEKTISKAKGQPREPQVYTLPPSQEEMTKNQVSLTCLVKGFYPSDIAVEWESNGQPENNYKTTPPVLDSDGSFFLYSRLTVDKSRWQEGNVFSCSVMHEALHNHYTQKSLSLSLG

SEQ ID NO: 84 - protein, 275 aa, Artificial Sequence
  GM-FI
HGEGTFTSDVSSYLEEQAAKEIIAWLVKGGGGGGGSGGGGSGGGGSAESKYGPPCPPCPAPEAAGGPSVFLFPPKPKDTLMISRTPEVTCVVVDVSQEDPEVQFNWYVDGVEVHNAKTKPREEQFNSTYRVVSVLTVLHQDWLNGKEYKCKVSNKGLPSSIEKTISKAKGQPREPQVYTLPPSQEEMTKNQVSLTCLVKGFYPSDIAVEWESNGQPENNYKTTPPVLDSDGSFFLYSRLTVDKSRWQEGNVFSCSVMHEALHNHYTQKSLSLSLG

SEQ ID NO: 85 - protein, 275 aa, Artificial Sequence
  GM-QN
HGEGTFTSDVSSYLEENAAKEFIAWLVKGGGGGGGSGGGGSGGGGSAESKYGPPCPPCPAPEAAGGPSVFLFPPKPKDTLMISRTPEVTCVVVDVSQEDPEVQFNWYVDGVEVHNAKTKPREEQFNSTYRVVSVLTVLHQDWLNGKEYKCKVSNKGLPSSIEKTISKAKGQPREPQVYTLPPSQEEMTKNQVSLTCLVKGFYPSDIAVEWESNGQPENNYKTTPPVLDSDGSFFLYSRLTVDKSRWQEGNVFSCSVMHEALHNHYTQKSLSLSLG

SEQ ID NO: 86 - protein, 275 aa, Artificial Sequence
  GM-QT
HGEGTFTSDVSSYLEETAAKEFIAWLVKGGGGGGGSGGGGSGGGGSAESKYGPPCPPCPAPEAAGGPSVFLFPPKPKDTLMISRTPEVTCVVVDVSQEDPEVQFNWYVDGVEVHNAKTKPREEQFNSTYRVVSVLTVLHQDWLNGKEYKCKVSNKGLPSSIEKTISKAKGQPREPQVYTLPPSQEEMTKNQVSLTCLVKGFYPSDIAVEWESNGQPENNYKTTPPVLDSDGSFFLYSRLTVDKSRWQEGNVFSCSVMHEALHNHYTQKSLSLSLG

SEQ ID NO: 87 - protein, 275 aa, Artificial Sequence
  GM-QS
HGEGTFTSDVSSYLEESAAKEFIAWLVKGGGGGGGSGGGGSGGGGSAESKYGPPCPPCPAPEAAGGPSVFLFPPKPKDTLMISRTPEVTCVVVDVSQEDPEVQFNWYVDGVEVHNAKTKPREEQFNSTYRVVSVLTVLHQDWLNGKEYKCKVSNKGLPSSIEKTISKAKGQPREPQVYTLPPSQEEMTKNQVSLTCLVKGFYPSDIAVEWESNGQPENNYKTTPPVLDSDGSFFLYSRLTVDKSRWQEGNVFSCSVMHEALHNHYTQKSLSLSLG

SEQ ID NO: 88 - protein, 275 aa, Artificial Sequence
  GM-QE
HGEGTFTSDVSSYLEEEAAKEFIAWLVKGGGGGGGSGGGGSGGGGSAESKYGPPCPPCPAPEAAGGPSVFLFPPKPKDTLMISRTPEVTCVVVDVSQEDPEVQFNWYVDGVEVHNAKTKPREEQFNSTYRVVSVLTVLHQDWLNGKEYKCKVSNKGLPSSIEKTISKAKGQPREPQVYTLPPSQEEMTKNQVSLTCLVKGFYPSDIAVEWESNGQPENNYKTTPPVLDSDGSFFLYSRLTVDKSRWQEGNVFSCSVMHEALHNHYTQKSLSLSLG

SEQ ID NO: 89 - protein, 275 aa, Artificial Sequence
  GM-YL
HGEGTFTSDVSSLLEEQAAKEFIAWLVKGGGGGGGSGGGGSGGGGSAESKYGPPCPPCPAPEAAGGPSVFLFPPKPKDTLMISRTPEVTCVVVDVSQEDPEVQFNWYVDGVEVHNAKTKPREEQFNSTYRVVSVLTVLHQDWLNGKEYKCKVSNKGLPSSIEKTISKAKGQPREPQVYTLPPSQEEMTKNQVSLTCLVKGFYPSDIAVEWESNGQPENNYKTTPPVLDSDGSFFLYSRLTVDKSRWQEGNVFSCSVMHEALHNHYTQKSLSLSLG

SEQ ID NO: 90 - protein, 275 aa, Artificial Sequence
  GM-YT
HGEGTFTSDVSSTLEEQAAKEFIAWLVKGGGGGGGSGGGGSGGGGSAESKYGPPCPPCPAPEAAGGPSVFLFPPKPKDTLMISRTPEVTCVVVDVSQEDPEVQFNWYVDGVEVHNAKTKPREEQFNSTYRVVSVLTVLHQDWLNGKEYKCKVSNKGLPSSIEKTISKAKGQPREPQVYTLPPSQEEMTKNQVSLTCLVKGFYPSDIAVEWESNGQPENNYKTTPPVLDSDGSFFLYSRLTVDKSRWQEGNVFSCSVMHEALHNHYTQKSLSLSLG

SEQ ID NO: 91 - protein, 275 aa, Artificial Sequence
  GM-YF
HGEGTFTSDVSSFLEEQAAKEFIAWLVKGGGGGGGSGGGGSGGGGSAESKYGPPCPPCPAPEAAGGPSVFLFPPKPKDTLMISRTPEVTCVVVDVSQEDPEVQFNWYVDGVEVHNAKTKPREEQFNSTYRVVSVLTVLHQDWLNGKEYKCKVSNKGLPSSIEKTISKAKGQPREPQVYTLPPSQEEMTKNQVSLTCLVKGFYPSDIAVEWESNGQPENNYKTTPPVLDSDGSFFLYSRLTVDKSRWQEGNVFSCSVMHEALHNHYTQKSLSLSLG

SEQ ID NO: 92 - protein, 275 aa, Artificial Sequence
  GM-YI
HGEGTFTSDVSSILEEQAAKEFIAWLVKGGGGGGGSGGGGSGGGGSAESKYGPPCPPCPAPEAAGGPSVFLFPPKPKDTLMISRTPEVTCVVVDVSQEDPEVQFNWYVDGVEVHNAKTKPREEQFNSTYRVVSVLTVLHQDWLNGKEYKCKVSNKGLPSSIEKTISKAKGQPREPQVYTLPPSQEEMTKNQVSLTCLVKGFYPSDIAVEWESNGQPENNYKTTPPVLDSDGSFFLYSRLTVDKSRWQEGNVFSCSVMHEALHNHYTQKSLSLSLG

SEQ ID NO: 93 - protein, 275 aa, Artificial Sequence
  GM-YV
HGEGTFTSDVSSVLEEQAAKEFIAWLVKGGGGGGGSGGGGSGGGGSAESKYGPPCPPCPAPEAAGGPSVFLFPPKPKDTLMISRTPEVTCVVVDVSQEDPEVQFNWYVDGVEVHNAKTKPREEQFNSTYRVVSVLTVLHQDWLNGKEYKCKVSNKGLPSSIEKTISKAKGQPREPQVYTLPPSQEEMTKNQVSLTCLVKGFYPSDIAVEWESNGQPENNYKTTPPVLDSDGSFFLYSRLTVDKSRWQEGNVFSCSVMHEALHNHYTQKSLSLSLG

SEQ ID NO: 94 - protein, 275 aa, Artificial Sequence
  GM-YS
HGEGTFTSDVSSSLEEQAAKEFIAWLVKGGGGGGGSGGGGSGGGGSAESKYGPPCPPCPAPEAAGGPSVFLFPPKPKDTLMISRTPEVTCVVVDVSQEDPEVQFNWYVDGVEVHNAKTKPREEQFNSTYRVVSVLTVLHQDWLNGKEYKCKVSNKGLPSSIEKTISKAKGQPREPQVYTLPPSQEEMTKNQVSLTCLVKGFYPSDIAVEWESNGQPENNYKTTPPVLDSDGSFFLYSRLTVDKSRWQEGNVFSCSVMHEALHNHYTQKSLSLSLG

SEQ ID NO: 95 - protein, 275 aa, Artificial Sequence
  GM-YA
HGEGTFTSDVSSALEEQAAKEFIAWLVKGGGGGGGSGGGGSGGGGSAESKYGPPCPPCPAPEAAGGPSVFLFPPKPKDTLMISRTPEVTCVVVDVSQEDPEVQFNWYVDGVEVHNAKTKPREEQFNSTYRVVSVLTVLHQDWLNGKEYKCKVSNKGLPSSIEKTISKAKGQPREPQVYTLPPSQEEMTKNQVSLTCLVKGFYPSDIAVEWESNGQPENNYKTTPPVLDSDGSFFLYSRLTVDKSRWQEGNVFSCSVMHEALHNHYTQKSLSLSLG

SEQ ID NO: 96 - protein, 275 aa, Artificial Sequence
  GM-KRWY
HGEGTFTSDVSSYLEEQAAREFIAYLVKGGGGGGGSGGGGSGGGGSAESKYGPPCPPCPAPEAAGGPSVFLFPPKPKDTLMISRTPEVTCVVVDVSQEDPEVQFNWYVDGVEVHNAKTKPREEQFNSTYRVVSVLTVLHQDWLNGKEYKCKVSNKGLPSSIEKTISKAKGQPREPQVYTLPPSQEEMTKNQVSLTCLVKGFYPSDIAVEWESNGQPENNYKTTPPVLDSDGSFFLYSRLTVDKSRWQEGNVFSCSVMHEALHNHYTQKSLSLSLG

SEQ ID NO: 97 - protein, 275 aa, Artificial Sequence
  GM-KRFY
HGEGTFTSDVSSYLEEQAAREYIAWLVKGGGGGGGSGGGGSGGGGSAESKYGPPCPPCPAPEAAGGPSVFLFPPKPKDTLMISRTPEVTCVVVDVSQEDPEVQFNWYVDGVEVHNAKTKPREEQFNSTYRVVSVLTVLHQDWLNGKEYKCKVSNKGLPSSIEKTISKAKGQPREPQVYTLPPSQEEMTKNQVSLTCLVKGFYPSDIAVEWESNGQPENNYKTTPPVLDSDGSFFLYSRLTVDKSRWQEGNVFSCSVMHEALHNHYTQKSLSLSLG

SEQ ID NO: 98 - protein, 275 aa, Artificial Sequence
  GM-KRWYFY
HGEGTFTSDVSSYLEEQAAREYIAYLVKGGGGGGGSGGGGSGGGGSAESKYGPPCPPCPAPEAAGGPSVFLFPPKPKDTLMISRTPEVTCVVVDVSQEDPEVQFNWYVDGVEVHNAKTKPREEQFNSTYRVVSVLTVLHQDWLNGKEYKCKVSNKGLPSSIEKTISKAKGQPREPQVYTLPPSQEEMTKNQVSLTCLVKGFYPSDIAVEWESNGQPENNYKTTPPVLDSDGSFFLYSRLTVDKSRWQEGNVFSCSVMHEALHNHYTQKSLSLSLG

SEQ ID NO: 99 - protein, 275 aa, Artificial Sequence
  GM-KRQN
HGEGTFTSDVSSYLEENAAREFIAWLVKGGGGGGGSGGGGSGGGGSAESKYGPPCPPCPAPEAAGGPSVFLFPPKPKDTLMISRTPEVTCVVVDVSQEDPEVQFNWYVDGVEVHNAKTKPREEQFNSTYRVVSVLTVLHQDWLNGKEYKCKVSNKGLPSSIEKTISKAKGQPREPQVYTLPPSQEEMTKNQVSLTCLVKGFYPSDIAVEWESNGQPENNYKTTPPVLDSDGSFFLYSRLTVDKSRWQEGNVFSCSVMHEALHNHYTQKSLSLSLG

SEQ ID NO: 100 - protein, 275 aa, Artificial Sequence
  GM-KRQT
HGEGTFTSDVSSYLEETAAREFIAWLVKGGGGGGGSGGGGSGGGGSAESKYGPPCPPCPAPEAAGGPSVFLFPPKPKDTLMISRTPEVTCVVVDVSQEDPEVQFNWYVDGVEVHNAKTKPREEQFNSTYRVVSVLTVLHQDWLNGKEYKCKVSNKGLPSSIEKTISKAKGQPREPQVYTLPPSQEEMTKNQVSLTCLVKGFYPSDIAVEWESNGQPENNYKTTPPVLDSDGSFFLYSRLTVDKSRWQEGNVFSCSVMHEALHNHYTQKSLSLSLG

SEQ ID NO: 101 - protein, 275 aa, Artificial Sequence
  GM-KRQS
HGEGTFTSDVSSYLEESAAREFIAWLVKGGGGGGGSGGGGSGGGGSAESKYGPPCPPCPAPEAAGGPSVFLFPPKPKDTLMISRTPEVTCVVVDVSQEDPEVQFNWYVDGVEVHNAKTKPREEQFNSTYRVVSVLTVLHQDWLNGKEYKCKVSNKGLPSSIEKTISKAKGQPREPQVYTLPPSQEEMTKNQVSLTCLVKGFYPSDIAVEWESNGQPENNYKTTPPVLDSDGSFFLYSRLTVDKSRWQEGNVFSCSVMHEALHNHYTQKSLSLSLG

SEQ ID NO: 102 - protein, 275 aa, Artificial Sequence
  GM-KRQE
HGEGTFTSDVSSYLEEEAAREFIAWLVKGGGGGGGSGGGGSGGGGSAESKYGPPCPPCPAPEAAGGPSVFLFPPKPKDTLMISRTPEVTCVVVDVSQEDPEVQFNWYVDGVEVHNAKTKPREEQFNSTYRVVSVLTVLHQDWLNGKEYKCKVSNKGLPSSIEKTISKAKGQPREPQVYTLPPSQEEMTKNQVSLTCLVKGFYPSDIAVEWESNGQPENNYKTTPPVLDSDGSFFLYSRLTVDKSRWQEGNVFSCSVMHEALHNHYTQKSLSLSLG

SEQ ID NO: 103 - protein, 275 aa, Artificial Sequence
  GM-KRYL
HGEGTFTSDVSSLLEEQAAREFIAWLVKGGGGGGGSGGGGSGGGGSAESKYGPPCPPCPAPEAAGGPSVFLFPPKPKDTLMISRTPEVTCVVVDVSQEDPEVQFNWYVDGVEVHNAKTKPREEQFNSTYRVVSVLTVLHQDWLNGKEYKCKVSNKGLPSSIEKTISKAKGQPREPQVYTLPPSQEEMTKNQVSLTCLVKGFYPSDIAVEWESNGQPENNYKTTPPVLDSDGSFFLYSRLTVDKSRWQEGNVFSCSVMHEALHNHYTQKSLSLSLG

SEQ ID NO: 104 - protein, 275 aa, Artificial Sequence
  GM-KRYT
HGEGTFTSDVSSTLEEQAAREFIAWLVKGGGGGGGSGGGGSGGGGSAESKYGPPCPPCPAPEAAGGPSVFLFPPKPKDTLMISRTPEVTCVVVDVSQEDPEVQFNWYVDGVEVHNAKTKPREEQFNSTYRVVSVLTVLHQDWLNGKEYKCKVSNKGLPSSIEKTISKAKGQPREPQVYTLPPSQEEMTKNQVSLTCLVKGFYPSDIAVEWESNGQPENNYKTTPPVLDSDGSFFLYSRLTVDKSRWQEGNVFSCSVMHEALHNHYTQKSLSLSLG

SEQ ID NO: 105 - protein, 275 aa, Artificial Sequence
  GM-KRYF
HGEGTFTSDVSSFLEEQAAREFIAWLVKGGGGGGGSGGGGSGGGGSAESKYGPPCPPCPAPEAAGGPSVFLFPPKPKDTLMISRTPEVTCVVVDVSQEDPEVQFNWYVDGVEVHNAKTKPREEQFNSTYRVVSVLTVLHQDWLNGKEYKCKVSNKGLPSSIEKTISKAKGQPREPQVYTLPPSQEEMTKNQVSLTCLVKGFYPSDIAVEWESNGQPENNYKTTPPVLDSDGSFFLYSRLTVDKSRWQEGNVFSCSVMHEALHNHYTQKSLSLSLG

SEQ ID NO: 106 - protein, 275 aa, Artificial Sequence
  GM-KRYI
HGEGTFTSDVSSILEEQAAREFIAWLVKGGGGGGGSGGGGSGGGGSAESKYGPPCPPCPAPEAAGGPSVFLFPPKPKDTLMISRTPEVTCVVVDVSQEDPEVQFNWYVDGVEVHNAKTKPREEQFNSTYRVVSVLTVLHQDWLNGKEYKCKVSNKGLPSSIEKTISKAKGQPREPQVYTLPPSQEEMTKNQVSLTCLVKGFYPSDIAVEWESNGQPENNYKTTPPVLDSDGSFFLYSRLTVDKSRWQEGNVFSCSVMHEALHNHYTQKSLSLSLG

SEQ ID NO: 107 - protein, 275 aa, Artificial Sequence
  GM-KRYV
HGEGTFTSDVSSVLEEQAAREFIAWLVKGGGGGGGSGGGGSGGGGSAESKYGPPCPPCPAPEAAGGPSVFLFPPKPKDTLMISRTPEVTCVVVDVSQEDPEVQFNWYVDGVEVHNAKTKPREEQFNSTYRVVSVLTVLHQDWLNGKEYKCKVSNKGLPSSIEKTISKAKGQPREPQVYTLPPSQEEMTKNQVSLTCLVKGFYPSDIAVEWESNGQPENNYKTTPPVLDSDGSFFLYSRLTVDKSRWQEGNVFSCSVMHEALHNHYTQKSLSLSLG

SEQ ID NO: 108 - protein, 275 aa, Artificial Sequence
  GM-KRYS
HGEGTFTSDVSSSLEEQAAREFIAWLVKGGGGGGGSGGGGSGGGGSAESKYGPPCPPCPAPEAAGGPSVFLFPPKPKDTLMISRTPEVTCVVVDVSQEDPEVQFNWYVDGVEVHNAKTKPREEQFNSTYRVVSVLTVLHQDWLNGKEYKCKVSNKGLPSSIEKTISKAKGQPREPQVYTLPPSQEEMTKNQVSLTCLVKGFYPSDIAVEWESNGQPENNYKTTPPVLDSDGSFFLYSRLTVDKSRWQEGNVFSCSVMHEALHNHYTQKSLSLSLG

SEQ ID NO: 109 - protein, 275 aa, Artificial Sequence
  GM-KRYA
HGEGTFTSDVSSALEEQAAREFIAWLVKGGGGGGGSGGGGSGGGGSAESKYGPPCPPCPAPEAAGGPSVFLFPPKPKDTLMISRTPEVTCVVVDVSQEDPEVQFNWYVDGVEVHNAKTKPREEQFNSTYRVVSVLTVLHQDWLNGKEYKCKVSNKGLPSSIEKTISKAKGQPREPQVYTLPPSQEEMTKNQVSLTCLVKGFYPSDIAVEWESNGQPENNYKTTPPVLDSDGSFFLYSRLTVDKSRWQEGNVFSCSVMHEALHNHYTQKSLSLSLG

SEQ ID NO: 110 - protein, 275 aa, Artificial Sequence
  GM-WYQN
HGEGTFTSDVSSYLEENAAKEFIAYLVKGGGGGGGSGGGGSGGGGSAESKYGPPCPPCPAPEAAGGPSVFLFPPKPKDTLMISRTPEVTCVVVDVSQEDPEVQFNWYVDGVEVHNAKTKPREEQFNSTYRVVSVLTVLHQDWLNGKEYKCKVSNKGLPSSIEKTISKAKGQPREPQVYTLPPSQEEMTKNQVSLTCLVKGFYPSDIAVEWESNGQPENNYKTTPPVLDSDGSFFLYSRLTVDKSRWQEGNVFSCSVMHEALHNHYTQKSLSLSLG

SEQ ID NO: 111 - protein, 275 aa, Artificial Sequence
  GM-WYQS
HGEGTFTSDVSSYLEESAAKEFIAYLVKGGGGGGGSGGGGSGGGGSAESKYGPPCPPCPAPEAAGGPSVFLFPPKPKDTLMISRTPEVTCVVVDVSQEDPEVQFNWYVDGVEVHNAKTKPREEQFNSTYRVVSVLTVLHQDWLNGKEYKCKVSNKGLPSSIEKTISKAKGQPREPQVYTLPPSQEEMTKNQVSLTCLVKGFYPSDIAVEWESNGQPENNYKTTPPVLDSDGSFFLYSRLTVDKSRWQEGNVFSCSVMHEALHNHYTQKSLSLSLG

SEQ ID NO: 112 - protein, 275 aa, Artificial Sequence
  GM-WYQT
HGEGTFTSDVSSYLEETAAKEFIAYLVKGGGGGGGSGGGGSGGGGSAESKYGPPCPPCPAPEAAGGPSVFLFPPKPKDTLMISRTPEVTCVVVDVSQEDPEVQFNWYVDGVEVHNAKTKPREEQFNSTYRVVSVLTVLHQDWLNGKEYKCKVSNKGLPSSIEKTISKAKGQPREPQVYTLPPSQEEMTKNQVSLTCLVKGFYPSDIAVEWESNGQPENNYKTTPPVLDSDGSFFLYSRLTVDKSRWQEGNVFSCSVMHEALHNHYTQKSLSLSLG

SEQ ID NO: 113 - protein, 275 aa, Artificial Sequence
  GM-WYQE
HGEGTFTSDVSSYLEEEAAKEFIAYLVKGGGGGGGSGGGGSGGGGSAESKYGPPCPPCPAPEAAGGPSVFLFPPKPKDTLMISRTPEVTCVVVDVSQEDPEVQFNWYVDGVEVHNAKTKPREEQFNSTYRVVSVLTVLHQDWLNGKEYKCKVSNKGLPSSIEKTISKAKGQPREPQVYTLPPSQEEMTKNQVSLTCLVKGFYPSDIAVEWESNGQPENNYKTTPPVLDSDGSFFLYSRLTVDKSRWQEGNVFSCSVMHEALHNHYTQKSLSLSLG

SEQ ID NO: 114 - protein, 275 aa, Artificial Sequence
  GM-WYYL
HGEGTFTSDVSSLLEEQAAKEFIAYLVKGGGGGGGSGGGGSGGGGSAESKYGPPCPPCPAPEAAGGPSVFLFPPKPKDTLMISRTPEVTCVVVDVSQEDPEVQFNWYVDGVEVHNAKTKPREEQFNSTYRVVSVLTVLHQDWLNGKEYKCKVSNKGLPSSIEKTISKAKGQPREPQVYTLPPSQEEMTKNQVSLTCLVKGFYPSDIAVEWESNGQPENNYKTTPPVLDSDGSFFLYSRLTVDKSRWQEGNVFSCSVMHEALHNHYTQKSLSLSLG

SEQ ID NO: 115 - protein, 275 aa, Artificial Sequence
  GM-WYYT
HGEGTFTSDVSSTLEEQAAKEFIAYLVKGGGGGGGSGGGGSGGGGSAESKYGPPCPPCPAPEAAGGPSVFLFPPKPKDTLMISRTPEVTCVVVDVSQEDPEVQFNWYVDGVEVHNAKTKPREEQFNSTYRVVSVLTVLHQDWLNGKEYKCKVSNKGLPSSIEKTISKAKGQPREPQVYTLPPSQEEMTKNQVSLTCLVKGFYPSDIAVEWESNGQPENNYKTTPPVLDSDGSFFLYSRLTVDKSRWQEGNVFSCSVMHEALHNHYTQKSLSLSLG

SEQ ID NO: 116 - protein, 275 aa, Artificial Sequence
  GM-WYYF
HGEGTFTSDVSSFLEEQAAKEFIAYLVKGGGGGGGSGGGGSGGGGSAESKYGPPCPPCPAPEAAGGPSVFLFPPKPKDTLMISRTPEVTCVVVDVSQEDPEVQFNWYVDGVEVHNAKTKPREEQFNSTYRVVSVLTVLHQDWLNGKEYKCKVSNKGLPSSIEKTISKAKGQPREPQVYTLPPSQEEMTKNQVSLTCLVKGFYPSDIAVEWESNGQPENNYKTTPPVLDSDGSFFLYSRLTVDKSRWQEGNVFSCSVMHEALHNHYTQKSLSLSLG

SEQ ID NO: 117 - protein, 275 aa, Artificial Sequence
  GM-WYYI
HGEGTFTSDVSSILEEQAAKEFIAYLVKGGGGGGGSGGGGSGGGGSAESKYGPPCPPCPAPEAAGGPSVFLFPPKPKDTLMISRTPEVTCVVVDVSQEDPEVQFNWYVDGVEVHNAKTKPREEQFNSTYRVVSVLTVLHQDWLNGKEYKCKVSNKGLPSSIEKTISKAKGQPREPQVYTLPPSQEEMTKNQVSLTCLVKGFYPSDIAVEWESNGQPENNYKTTPPVLDSDGSFFLYSRLTVDKSRWQEGNVFSCSVMHEALHNHYTQKSLSLSLG

SEQ ID NO: 118 - protein, 275 aa, Artificial Sequence
  GM-WYYV
HGEGTFTSDVSSVLEEQAAKEFIAYLVKGGGGGGGSGGGGSGGGGSAESKYGPPCPPCPAPEAAGGPSVFLFPPKPKDTLMISRTPEVTCVVVDVSQEDPEVQFNWYVDGVEVHNAKTKPREEQFNSTYRVVSVLTVLHQDWLNGKEYKCKVSNKGLPSSIEKTISKAKGQPREPQVYTLPPSQEEMTKNQVSLTCLVKGFYPSDIAVEWESNGQPENNYKTTPPVLDSDGSFFLYSRLTVDKSRWQEGNVFSCSVMHEALHNHYTQKSLSLSLG

SEQ ID NO: 119 - protein, 275 aa, Artificial Sequence
  GM-WYYS
HGEGTFTSDVSSSLEEQAAKEFIAYLVKGGGGGGGSGGGGSGGGGSAESKYGPPCPPCPAPEAAGGPSVFLFPPKPKDTLMISRTPEVTCVVVDVSQEDPEVQFNWYVDGVEVHNAKTKPREEQFNSTYRVVSVLTVLHQDWLNGKEYKCKVSNKGLPSSIEKTISKAKGQPREPQVYTLPPSQEEMTKNQVSLTCLVKGFYPSDIAVEWESNGQPENNYKTTPPVLDSDGSFFLYSRLTVDKSRWQEGNVFSCSVMHEALHNHYTQKSLSLSLG

SEQ ID NO: 120 - protein, 275 aa, Artificial Sequence
  GM-WYYA
HGEGTFTSDVSSALEEQAAKEFIAYLVKGGGGGGGSGGGGSGGGGSAESKYGPPCPPCPAPEAAGGPSVFLFPPKPKDTLMISRTPEVTCVVVDVSQEDPEVQFNWYVDGVEVHNAKTKPREEQFNSTYRVVSVLTVLHQDWLNGKEYKCKVSNKGLPSSIEKTISKAKGQPREPQVYTLPPSQEEMTKNQVSLTCLVKGFYPSDIAVEWESNGQPENNYKTTPPVLDSDGSFFLYSRLTVDKSRWQEGNVFSCSVMHEALHNHYTQKSLSLSLG

SEQ ID NO: 121 - protein, 275 aa, Artificial Sequence
  GM-WYFY
HGEGTFTSDVSSYLEEQAAKEYIAYLVKGGGGGGGSGGGGSGGGGSAESKYGPPCPPCPAPEAAGGPSVFLFPPKPKDTLMISRTPEVTCVVVDVSQEDPEVQFNWYVDGVEVHNAKTKPREEQFNSTYRVVSVLTVLHQDWLNGKEYKCKVSNKGLPSSIEKTISKAKGQPREPQVYTLPPSQEEMTKNQVSLTCLVKGFYPSDIAVEWESNGQPENNYKTTPPVLDSDGSFFLYSRLTVDKSRWQEGNVFSCSVMHEALHNHYTQKSLSLSLG

SEQ ID NO: 122 - protein, 275 aa, Artificial Sequence
  GM-WYFL
HGEGTFTSDVSSYLEEQAAKELIAYLVKGGGGGGGSGGGGSGGGGSAESKYGPPCPPCPAPEAAGGPSVFLFPPKPKDTLMISRTPEVTCVVVDVSQEDPEVQFNWYVDGVEVHNAKTKPREEQFNSTYRVVSVLTVLHQDWLNGKEYKCKVSNKGLPSSIEKTISKAKGQPREPQVYTLPPSQEEMTKNQVSLTCLVKGFYPSDIAVEWESNGQPENNYKTTPPVLDSDGSFFLYSRLTVDKSRWQEGNVFSCSVMHEALHNHYTQKSLSLSLG

SEQ ID NO: 123 - protein, 275 aa, Artificial Sequence
  GM-WA
HGEGTFTSDVSSYLEEQAAKEFIAALVKGGGGGGGSGGGGSGGGGSAESKYGPPCPPCPAPEAAGGPSVFLFPPKPKDTLMISRTPEVTCVVVDVSQEDPEVQFNWYVDGVEVHNAKTKPREEQFNSTYRVVSVLTVLHQDWLNGKEYKCKVSNKGLPSSIEKTISKAKGQPREPQVYTLPPSQEEMTKNQVSLTCLVKGFYPSDIAVEWESNGQPENNYKTTPPVLDSDGSFFLYSRLTVDKSRWQEGNVFSCSVMHEALHNHYTQKSLSLSLG

SEQ ID NO: 124 - protein, 275 aa, Artificial Sequence
  GM-WL
HGEGTFTSDVSSYLEEQAAKEFIALLVKGGGGGGGSGGGGSGGGGSAESKYGPPCPPCPAPEAAGGPSVFLFPPKPKDTLMISRTPEVTCVVVDVSQEDPEVQFNWYVDGVEVHNAKTKPREEQFNSTYRVVSVLTVLHQDWLNGKEYKCKVSNKGLPSSIEKTISKAKGQPREPQVYTLPPSQEEMTKNQVSLTCLVKGFYPSDIAVEWESNGQPENNYKTTPPVLDSDGSFFLYSRLTVDKSRWQEGNVFSCSVMHEALHNHYTQKSLSLSLG

SEQ ID NO: 125 - protein, 275 aa, Artificial Sequence
  GM-FL
HGEGTFTSDVSSYLEEQAAKELIAWLVKGGGGGGGSGGGGSGGGGSAESKYGPPCPPCPAPEAAGGPSVFLFPPKPKDTLMISRTPEVTCVVVDVSQEDPEVQFNWYVDGVEVHNAKTKPREEQFNSTYRVVSVLTVLHQDWLNGKEYKCKVSNKGLPSSIEKTISKAKGQPREPQVYTLPPSQEEMTKNQVSLTCLVKGFYPSDIAVEWESNGQPENNYKTTPPVLDSDGSFFLYSRLTVDKSRWQEGNVFSCSVMHEALHNHYTQKSLSLSLG

SEQ ID NO: 126 - protein, 275 aa, Artificial Sequence
  GM-WIFL
HGEGTFTSDVSSYLEEQAAKELIAILVKGGGGGGGSGGGGSGGGGSAESKYGPPCPPCPAPEAAGGPSVFLFPPKPKDTLMISRTPEVTCVVVDVSQEDPEVQFNWYVDGVEVHNAKTKPREEQFNSTYRVVSVLTVLHQDWLNGKEYKCKVSNKGLPSSIEKTISKAKGQPREPQVYTLPPSQEEMTKNQVSLTCLVKGFYPSDIAVEWESNGQPENNYKTTPPVLDSDGSFFLYSRLTVDKSRWQEGNVFSCSVMHEALHNHYTQKSLSLSLG

SEQ ID NO: 127 - protein, 275 aa, Artificial Sequence
  GM-WLFL
HGEGTFTSDVSSYLEEQAAKELIALLVKGGGGGGGSGGGGSGGGGSAESKYGPPCPPCPAPEAAGGPSVFLFPPKPKDTLMISRTPEVTCVVVDVSQEDPEVQFNWYVDGVEVHNAKTKPREEQFNSTYRVVSVLTVLHQDWLNGKEYKCKVSNKGLPSSIEKTISKAKGQPREPQVYTLPPSQEEMTKNQVSLTCLVKGFYPSDIAVEWESNGQPENNYKTTPPVLDSDGSFFLYSRLTVDKSRWQEGNVFSCSVMHEALHNHYTQKSLSLSLG

SEQ ID NO: 128 - protein, 275 aa, Artificial Sequence
  GM-KRWYQN
HGEGTFTSDVSSYLEENAAREFIAYLVKGGGGGGGSGGGGSGGGGSAESKYGPPCPPCPAPEAAGGPSVFLFPPKPKDTLMISRTPEVTCVVVDVSQEDPEVQFNWYVDGVEVHNAKTKPREEQFNSTYRVVSVLTVLHQDWLNGKEYKCKVSNKGLPSSIEKTISKAKGQPREPQVYTLPPSQEEMTKNQVSLTCLVKGFYPSDIAVEWESNGQPENNYKTTPPVLDSDGSFFLYSRLTVDKSRWQEGNVFSCSVMHEALHNHYTQKSLSLSLG

SEQ ID NO: 129 - protein, 275 aa, Artificial Sequence
  GM-KRWYQT
HGEGTFTSDVSSYLEETAAREFIAYLVKGGGGGGGSGGGGSGGGGSAESKYGPPCPPCPAPEAAGGPSVFLFPPKPKDTLMISRTPEVTCVVVDVSQEDPEVQFNWYVDGVEVHNAKTKPREEQFNSTYRVVSVLTVLHQDWLNGKEYKCKVSNKGLPSSIEKTISKAKGQPREPQVYTLPPSQEEMTKNQVSLTCLVKGFYPSDIAVEWESNGQPENNYKTTPPVLDSDGSFFLYSRLTVDKSRWQEGNVFSCSVMHEALHNHYTQKSLSLSLG

SEQ ID NO: 130 - protein, 275 aa, Artificial Sequence
  GM-KRWYQS
HGEGTFTSDVSSYLEESAAREFIAYLVKGGGGGGGSGGGGSGGGGSAESKYGPPCPPCPAPEAAGGPSVFLFPPKPKDTLMISRTPEVTCVVVDVSQEDPEVQFNWYVDGVEVHNAKTKPREEQFNSTYRVVSVLTVLHQDWLNGKEYKCKVSNKGLPSSIEKTISKAKGQPREPQVYTLPPSQEEMTKNQVSLTCLVKGFYPSDIAVEWESNGQPENNYKTTPPVLDSDGSFFLYSRLTVDKSRWQEGNVFSCSVMHEALHNHYTQKSLSLSLG

SEQ ID NO: 131 - protein, 275 aa, Artificial Sequence
  GM-KRWYQE
HGEGTFTSDVSSYLEEEAAREFIAYLVKGGGGGGGSGGGGSGGGGSAESKYGPPCPPCPAPEAAGGPSVFLFPPKPKDTLMISRTPEVTCVVVDVSQEDPEVQFNWYVDGVEVHNAKTKPREEQFNSTYRVVSVLTVLHQDWLNGKEYKCKVSNKGLPSSIEKTISKAKGQPREPQVYTLPPSQEEMTKNQVSLTCLVKGFYPSDIAVEWESNGQPENNYKTTPPVLDSDGSFFLYSRLTVDKSRWQEGNVFSCSVMHEALHNHYTQKSLSLSLG

SEQ ID NO: 132 - protein, 275 aa, Artificial Sequence
  GM-KRWYYF
HGEGTFTSDVSSFLEEQAAREFIAYLVKGGGGGGGSGGGGSGGGGSAESKYGPPCPPCPAPEAAGGPSVFLFPPKPKDTLMISRTPEVTCVVVDVSQEDPEVQFNWYVDGVEVHNAKTKPREEQFNSTYRVVSVLTVLHQDWLNGKEYKCKVSNKGLPSSIEKTISKAKGQPREPQVYTLPPSQEEMTKNQVSLTCLVKGFYPSDIAVEWESNGQPENNYKTTPPVLDSDGSFFLYSRLTVDKSRWQEGNVFSCSVMHEALHNHYTQKSLSLSLG

SEQ ID NO: 133 - protein, 275 aa, Artificial Sequence
  GM-KRWYYL
HGEGTFTSDVSSLLEEQAAREFIAYLVKGGGGGGGSGGGGSGGGGSAESKYGPPCPPCPAPEAAGGPSVFLFPPKPKDTLMISRTPEVTCVVVDVSQEDPEVQFNWYVDGVEVHNAKTKPREEQFNSTYRVVSVLTVLHQDWLNGKEYKCKVSNKGLPSSIEKTISKAKGQPREPQVYTLPPSQEEMTKNQVSLTCLVKGFYPSDIAVEWESNGQPENNYKTTPPVLDSDGSFFLYSRLTVDKSRWQEGNVFSCSVMHEALHNHYTQKSLSLSLG

SEQ ID NO: 134 - protein, 275 aa, Artificial Sequence
  GM-KRWYYT
HGEGTFTSDVSSTLEEQAAREFIAYLVKGGGGGGGSGGGGSGGGGSAESKYGPPCPPCPAPEAAGGPSVFLFPPKPKDTLMISRTPEVTCVVVDVSQEDPEVQFNWYVDGVEVHNAKTKPREEQFNSTYRVVSVLTVLHQDWLNGKEYKCKVSNKGLPSSIEKTISKAKGQPREPQVYTLPPSQEEMTKNQVSLTCLVKGFYPSDIAVEWESNGQPENNYKTTPPVLDSDGSFFLYSRLTVDKSRWQEGNVFSCSVMHEALHNHYTQKSLSLSLG

SEQ ID NO: 135 - protein, 275 aa, Artificial Sequence
  GM-KRWYYI
HGEGTFTSDVSSILEEQAAREFIAYLVKGGGGGGGSGGGGSGGGGSAESKYGPPCPPCPAPEAAGGPSVFLFPPKPKDTLMISRTPEVTCVVVDVSQEDPEVQFNWYVDGVEVHNAKTKPREEQFNSTYRVVSVLTVLHQDWLNGKEYKCKVSNKGLPSSIEKTISKAKGQPREPQVYTLPPSQEEMTKNQVSLTCLVKGFYPSDIAVEWESNGQPENNYKTTPPVLDSDGSFFLYSRLTVDKSRWQEGNVFSCSVMHEALHNHYTQKSLSLSLG

SEQ ID NO: 136 - protein, 275 aa, Artificial Sequence
  GM-KRWYYV
HGEGTFTSDVSSVLEEQAAREFIAYLVKGGGGGGGSGGGGSGGGGSAESKYGPPCPPCPAPEAAGGPSVFLFPPKPKDTLMISRTPEVTCVVVDVSQEDPEVQFNWYVDGVEVHNAKTKPREEQFNSTYRVVSVLTVLHQDWLNGKEYKCKVSNKGLPSSIEKTISKAKGQPREPQVYTLPPSQEEMTKNQVSLTCLVKGFYPSDIAVEWESNGQPENNYKTTPPVLDSDGSFFLYSRLTVDKSRWQEGNVFSCSVMHEALHNHYTQKSLSLSLG

SEQ ID NO: 137 - protein, 275 aa, Artificial Sequence
  GM-KRWYYS
HGEGTFTSDVSSSLEEQAAREFIAYLVKGGGGGGGSGGGGSGGGGSAESKYGPPCPPCPAPEAAGGPSVFLFPPKPKDTLMISRTPEVTCVVVDVSQEDPEVQFNWYVDGVEVHNAKTKPREEQFNSTYRVVSVLTVLHQDWLNGKEYKCKVSNKGLPSSIEKTISKAKGQPREPQVYTLPPSQEEMTKNQVSLTCLVKGFYPSDIAVEWESNGQPENNYKTTPPVLDSDGSFFLYSRLTVDKSRWQEGNVFSCSVMHEALHNHYTQKSLSLSLG

SEQ ID NO: 138 - protein, 275 aa, Artificial Sequence
  GM-KRWYYA
HGEGTFTSDVSSALEEQAAREFIAYLVKGGGGGGGSGGGGSGGGGSAESKYGPPCPPCPAPEAAGGPSVFLFPPKPKDTLMISRTPEVTCVVVDVSQEDPEVQFNWYVDGVEVHNAKTKPREEQFNSTYRVVSVLTVLHQDWLNGKEYKCKVSNKGLPSSIEKTISKAKGQPREPQVYTLPPSQEEMTKNQVSLTCLVKGFYPSDIAVEWESNGQPENNYKTTPPVLDSDGSFFLYSRLTVDKSRWQEGNVFSCSVMHEALHNHYTQKSLSLSLG

SEQ ID NO: 139 - protein, 232 aa, Homo sapiens
EPKSCDKTHTCPPCPAPELLGGPSVFLFPPKPKDTLMISRTPEVTCVVVDVSHEDPEVKFNWYVDGVEVHNAKTKPREEQYNSTYRVVSVLTVLHQDWLNGKEYKCKVSNKALPAPIEKTISKAKGQPREPQVYTLPPSRDELTKNQVSLTCLVKGFYPSDIAVEWESNGQPENNYKTTPPVLDSDGSFFLYSKLTVDKSRWQQGNVFSCSVMHEALHNHYTQKSLSLSPGK

SEQ ID NO: 140 - protein, 228 aa, Homo sapiens
ERKCCVECPPCPAPPVAGPSVFLFPPKPKDTLMISRTPEVTCVVVDVSHEDPEVQFNWYVDGVEVHNAKTKPREEQFNSTFRVVSVLTVVHQDWLNGKEYKCKVSNKGLPAPIEKTISKTKGQPREPQVYTLPPSREEMTKNQVSLTCLVKGFYPSDISVEWESNGQPENNYKTTPPMLDSDGSFFLYSKLTVDKSRWQQGNVFSCSVMHEALHNHYTQKSLSLSPGK

SEQ ID NO: 141 - protein, 232 aa, Homo sapiens
EPKSCDTPPPCPRCPAPELLGGPSVFLFPPKPKDTLMISRTPEVTCVVVDVSHEDPEVQFKWYVDGVEVHNAKTKPREEQYNSTFRVVSVLTVLHQDWLNGKEYKCKVSNKALPAPIEKTISKTKGQPREPQVYTLPPSREEMTKNQVSLTCLVKGFYPSDIAVEWESSGQPENNYNTTPPMLDSDGSFFLYSKLTVDKSRWQQGNIFSCSVMHEALHNRFTQKSLSLSPGK

SEQ ID NO: 142 - protein, 229 aa, Homo sapiens
ESKYGPPCPSCPAPEFLGGPSVFLFPPKPKDTLMISRTPEVTCVVVDVSQEDPEVQFNWYVDGVEVHNAKTKPREEQFNSTYRVVSVLTVLHQDWLNGKEYKCKVSNKGLPSSIEKTISKAKGQPREPQVYTLPPSQEEMTKNQVSLTCLVKGFYPSDIAVEWESNGQPENNYKTTPPVLDSDGSFFLYSRLTVDKSRWQEGNVFSCSVMHEALHNHYTQKSLSLSLGK

SEQ ID NO: 143 - protein, 229 aa, Artificial Sequence
  Fc of dulaglutide
AESKYGPPCPPCPAPEAAGGPSVFLFPPKPKDTLMISRTPEVTCVVVDVSQEDPEVQFNWYVDGVEVHNAKTKPREEQFNSTYRVVSVLTVLHQDWLNGKEYKCKVSNKGLPSSIEKTISKAKGQPREPQVYTLPPSQEEMTKNQVSLTCLVKGFYPSDIAVEWESNGQPENNYKTTPPVLDSDGSFFLYSRLTVDKSRWQEGNVFSCSVMHEALHNHYTQKSLSLSLG

SEQ ID NO: 144 - protein, 2 aa, Artificial Sequence
  GS linker peptide
GS

SEQ ID NO: 145 - protein, 3 aa, Artificial Sequence
  GAP linker peptide
GAP

SEQ ID NO: 146 - protein, 5 aa, Artificial Sequence
  G4S linker peptide
GGGGS

SEQ ID NO: 147 - protein, 10 aa, Artificial Sequence
  (G4S)2 linker peptide
GGGGSGGGGS

SEQ ID NO: 148 - protein, 15 aa, Artificial Sequence
  (G4S)3 linker peptide
GGGGSGGGGSGGGGS

SEQ ID NO: 149 - protein, 20 aa, Artificial Sequence
  (G4S)4 linker peptide
GGGGSGGGGSGGGGSGGGGS

SEQ ID NO: 150 - protein, 31 aa, Artificial Sequence
  GLP-1 variant general formula 2
  X19 (13)..(13): X19 may be Y, A, L, T, F, I, V or S
  X23 (17)..(17): X23 may be Q, E, T, S or N
HGEGTFTSDVSSXLEEXAAREFIAYLVKGGG

SEQ ID NO: 151 - protein, 31 aa, Artificial Sequence
  GLP-1 variant general formula 3
  X23 (17)..(17): X23 may be Q, E, T, S or N
HGEGTFTSDVSSYLEEXAAREFIAYLVKGGG

SEQ ID NO: 152 - protein, 31 aa, Artificial Sequence
  GLP-1 variant general formula 4
  X19 (13)..(13): X19 may be Y, A, L, T, F, I, V or S
HGEGTFTSDVSSXLEEQAAREFIAYLVKGGG

SEQ ID NO: 153 - protein, 31 aa, Artificial Sequence
  GLP-1 variant general formula 1
  X19 (13)..(13): X19 may be Y, A, L, T, F, I, V or S
  X23 (17)..(17): X23 may be Q, E, T, S or N
  X26 (20)..(20): X26 may be K or R
  X31 (25)..(25): X31 may be W, Y, K, R or A
HGEGTFTSDVSSXLEEXAAXEFIAXLVKGGG

SEQ ID NO: 154 - protein, 31 aa, Artificial Sequence
  GLP-1-KAWA
HGEGTFTSDVSSYLEEQAAAEFIAALVKGGG